European Patent Specification EP 4 284 942 B1, published August 14, 2024. Title: METHOD FOR TRANSPOSASE MEDIATED SPATIAL TAGGING AND ANALYZING GENOMIC DNA IN A BIOLOGICAL SAMPLE. Applicant: 10x Genomics, Inc. The sequence listing filed with the application follows.

SEQUENCE LISTING (13 sequences)

SEQ ID NO: 1 - protein, 476 aa, Escherichia coli
MITSALHRAADWAKSVFSSAALGDPRRTARLVNVAAQLAKYSGKSITISSEGSEAMQEGAYRFIRNPNVSAEAIRKAGAMQTVKLAQEFPELLAIEDTTSLSYRHQVAEELGKLGSIQDKSRGWWVHSVLLLEATTFRTVGLLHQEWWMRPDDPADADEKESGKWLAAAATSRLRMGSMMSNVIAVCDREADIHAYLQDKLAHNERFVVRSKHPRKDVESGLYLYDHLKNQPELGGYQISIPQKGVVDKRGKRKNRPARKASLSLRSGRITLKQGNITLNAVLAEEINPPKGETPLKWLLLTSEPVESLAQALRVIDIYTHRWRIEEFHKAWKTGAGAERQRMEEPDNLERMVSILSFVAVRLLQLRESFTLPQALRAQGLLKEAEHVESQSAETVLTPDECQLLGYLDKGKRKRKEKAGSLQWAYMAIARLGGFMDSKRTGIASWGALWEGWEALQSKLDGFLAAKDLMAQGIKI

SEQ ID NO: 2 - DNA, 19 bp, Artificial
  Tn5 Mosaic End Sequence
ctgtctcttatacacatct

SEQ ID NO: 3 - protein, 662 aa, Bacteriophage Mu
MKEWYTAKELLGLAGLPKQATNITRKAQREGWEFRQVAGTKGVSFEFNIKSFPVALRAEILLQQGRIETSQGYFEIARPTLEAHDYDREALWSKWDNASDSQRRLAEKWLPAVQAADEMLNQGISTKTAFATVAGHYQVSASTLRDKYYQVQKFAKPDWAAALVDGRGASRRNVHKSEFDEDAWQFLIADYLRPEKPAFRKCYERLELAAREHGWSIPSRATAFRRIQQLDEAMVVACREGEHALMHLIPAQQRTVEHLDAMQWINGDGYLHNVFVRWFNGDVIRPKTWFWQDVKTRKILGWRCDVSENIDSIRLSFMDVVTRYGIPEDFHITIDNTRGAANKWLTGGAPNRYRFKVKEDDPKGLFLLMGAKMHWTSVVAGKGWGQAKPVERAFGVGGLEEYVDKHPALAGAYTGPNPQAKPDNYGDRAVDAELFLKTLAEGVAMFNARTGRETEMCGGKLSFDDVFEREYARTIVRKPTEEQKRMLLLPAEAVNVSRKGEFALKVGGSLKGAKNVYYNMALMNAGVKKVVVRFDPQQLHSTVYCYTLDGRFICEAECLAPVAFNDAAAGREYRRRQKQLKSATKAAIKAQKQMDALEVAELLPQIAEPEAPESRIVGIFRPSGNTERVKNQERDDEYETERDEYLNHSLDILEQNRRKKAI

SEQ ID NO: 4 - DNA, 27 bp, Artificial
  Mu Transposase Recognition Sequence
tgaagcggcgcacgaaaaacgcgaaag

SEQ ID NO: 5 - DNA, 23 bp, Artificial
  Mu Transposase Recognition Sequence
gcgtttcacgataaatgcgaaaa

SEQ ID NO: 6 - DNA, 23 bp, Artificial
  Mu Transposase Recognition Sequence
ctgtttcatttgaagcgcgaaag

SEQ ID NO: 7 - DNA, 27 bp, Artificial
  Mu Transposase Recognition Sequence
tgtattgattcacttgaagtacgaaaa

SEQ ID NO: 8 - DNA, 23 bp, Artificial
  Mu Transposase Recognition Sequence
ccttaatcaatgaaacgcgaaag

SEQ ID NO: 9 - DNA, 23 bp, Artificial
  Mu Transposase Recognition Sequence
ttgtttcattgaaaatacgaaaa

SEQ ID NO: 10 - protein, 458 aa, Vibrio harveyi
MTHSDAKLWAQEQFGQAQLKDPRRTQRLISLATSIANQPGVSVAKLPFSPADMEGAYRFIRNENINAEDIAEAGFQSTVSRANEHKELLALEDTTTLSFPHRSIKEELGHTNQGDRTRALHVHSTLLFAPQSQTIVGLIEQQRWSEDITKRGQKHQHATRPYKEKESYKWEQASRRVVERLGDKMLDVISVCDREADLFEYLTYKRQHQQRFVVRSMQSRCLEEHAQKLYDYAQALPSVETKALTIPQKGGRKARNVKLDVKYGQVTLKAPANKKEHAGIPVYYVGCLEQGTSKDLAWHLLTSEPINNVDDAMRIIGYYERRWLIEDFHKVWKSEGTDVESLRLQSKDNLERLSVIYAFVATRLLALRFMKEVDELTKESCEKVLGQKAWKLLWLKLESKTLPKEVPDMGWAYKNLAKLGGWKDTKRTGRASIKVLWEGWFKLQTILEGYELAMSLDH

SEQ ID NO: 11 - DNA, 19 bp, Artificial
  V. harveyi Transposase Recognition Sequence
ctgtctcttgatcacaagt

SEQ ID NO: 12 - DNA, 19 bp, Artificial
  V. harveyi Transposase Recognition Sequence
agatgtgatcaagagacag

SEQ ID NO: 13 - DNA, 19 bp, Artificial
  V. harveyi Transposase Recognition Sequence
ctgtctcttgatcacatct